European Patent Application EP 4 786 485 A1, published August 5, 2026. Title: 直链肽化合物及其应用. Applicant: 深圳众格生物科技有限公司. The sequence listing filed with the application follows.

SEQUENCE LISTING (433 sequences)

SEQ ID NO: 1 - protein, 9 aa, synthetic construct
  VARIANT 1: note = ACE
  VARIANT 5: note = P01
  VARIANT 9: note = NME
XGHKXGHKX

SEQ ID NO: 2 - protein, 9 aa, synthetic construct
  VARIANT 1: note = ACE
  VARIANT 5: note = P02
  VARIANT 9: note = NME
XGHKXGHKX

SEQ ID NO: 3 - protein, 9 aa, synthetic construct
  VARIANT 1: note = ACE
  VARIANT 5: note = P03
  VARIANT 9: note = NME
XGHKXGHKX

SEQ ID NO: 4 - protein, 9 aa, synthetic construct
  VARIANT 1: note = ACE
  VARIANT 5: note = P04
  VARIANT 9: note = NME
XGHKXGHKX

SEQ ID NO: 5 - protein, 9 aa, synthetic construct
  VARIANT 1: note = ACE
  VARIANT 5: note = P05
  VARIANT 9: note = NME
XGHKXGHKX

SEQ ID NO: 6 - protein, 9 aa, synthetic construct
  VARIANT 1: note = ACE
  VARIANT 5: note = P06
  VARIANT 9: note = NME
XGHKXGHKX

SEQ ID NO: 7 - protein, 9 aa, synthetic construct
  VARIANT 1: note = ACE
  VARIANT 5: note = P07
  VARIANT 9: note = NME
XGHKXGHKX

SEQ ID NO: 8 - protein, 9 aa, synthetic construct
  VARIANT 1: note = ACE
  VARIANT 5: note = P08
  VARIANT 9: note = NME
XGHKXGHKX

SEQ ID NO: 9 - protein, 9 aa, synthetic construct
  VARIANT 1: note = ACE
  VARIANT 5: note = P09
  VARIANT 9: note = NME
XGHKXGHKX

SEQ ID NO: 10 - protein, 9 aa, synthetic construct
  VARIANT 1: note = ACE
  VARIANT 5: note = P10
  VARIANT 9: note = NME
XGHKXGHKX

SEQ ID NO: 11 - protein, 9 aa, synthetic construct
  VARIANT 1: note = ACE
  VARIANT 5: note = P11
  VARIANT 9: note = NME
XGHKXGHKX

SEQ ID NO: 12 - protein, 9 aa, synthetic construct
  VARIANT 1: note = ACE
  VARIANT 5: note = P12
  VARIANT 9: note = NME
XGHKXGHKX

SEQ ID NO: 13 - protein, 9 aa, synthetic construct
  VARIANT 1: note = ACE
  VARIANT 5: note = P13
  VARIANT 9: note = NME
XGHKXGHKX

SEQ ID NO: 14 - protein, 9 aa, synthetic construct
  VARIANT 1: note = ACE
  VARIANT 5: note = P14
  VARIANT 9: note = NME
XGHKXGHKX

SEQ ID NO: 15 - protein, 9 aa, synthetic construct
  VARIANT 1: note = ACE
  VARIANT 5: note = P15
  VARIANT 9: note = NME
XGHKXGHKX

SEQ ID NO: 16 - protein, 9 aa, synthetic construct
  VARIANT 1: note = ACE
  VARIANT 5: note = P16
  VARIANT 9: note = NME
XGHKXGHKX

SEQ ID NO: 17 - protein, 9 aa, synthetic construct
  VARIANT 1: note = ACE
  VARIANT 5: note = P17
  VARIANT 9: note = NME
XGHKXGHKX

SEQ ID NO: 18 - protein, 9 aa, synthetic construct
  VARIANT 1: note = ACE
  VARIANT 5: note = P18
  VARIANT 9: note = NME
XGHKXGHKX

SEQ ID NO: 19 - protein, 10 aa, synthetic construct
  VARIANT 1: note = ACE
  VARIANT 10: note = NME
XGHKGGGHKX

SEQ ID NO: 20 - protein, 11 aa, synthetic construct
  VARIANT 1: note = ACE
  VARIANT 11: note = NME
XGHKGGGGHKX

SEQ ID NO: 21 - protein, 9 aa, synthetic construct
  VARIANT 1: note = ACE
  VARIANT 5: note = P21
  VARIANT 9: note = NME
XGHKXGHKX

SEQ ID NO: 22 - protein, 10 aa, synthetic construct
  VARIANT 1: note = ACE
  VARIANT 10: note = NME
XGHKAAGHKX

SEQ ID NO: 23 - protein, 11 aa, synthetic construct
  VARIANT 1: note = ACE
  VARIANT 11: note = NME
XGHKAAAGHKX

SEQ ID NO: 24 - protein, 10 aa, synthetic construct
  VARIANT 1: note = ACE
  VARIANT 10: note = NME
XGHKPPGHKX

SEQ ID NO: 25 - protein, 11 aa, synthetic construct
  VARIANT 1: note = ACE
  VARIANT 11: note = NME
XGHKPPPGHKX

SEQ ID NO: 26 - protein, 9 aa, synthetic construct
  VARIANT 1: note = ACE
  VARIANT 5: note = P26
  VARIANT 9: note = NME
XGHKXGHKX

SEQ ID NO: 27 - protein, 9 aa, synthetic construct
  VARIANT 1: note = ACE
  VARIANT 5: note = P27
  VARIANT 9: note = NME
XGHKXGHKX

SEQ ID NO: 28 - protein, 9 aa, synthetic construct
  VARIANT 1: note = ACE
  VARIANT 5: note = P28
  VARIANT 9: note = NME
XGHKXGHKX

SEQ ID NO: 29 - protein, 9 aa, synthetic construct
  VARIANT 1: note = ACE
  VARIANT 5: note = P29
  VARIANT 9: note = NME
XGHKXGHKX

SEQ ID NO: 30 - protein, 9 aa, synthetic construct
  VARIANT 1: note = ACE
  VARIANT 5: note = P30
  VARIANT 9: note = NME
XGHKXGHKX

SEQ ID NO: 31-33 - skipped (3 entries)

SEQ ID NO: 34 - protein, 8 aa, synthetic construct
  VARIANT 1: note = ACE
  VARIANT 8: note = NME
XAAAGHKX

SEQ ID NO: 35-39 - skipped (5 entries)

SEQ ID NO: 40 - protein, 8 aa, synthetic construct
  VARIANT 1: note = ACE
  VARIANT 8: note = NME
XGGGGHKX

SEQ ID NO: 41-43 - skipped (3 entries)

SEQ ID NO: 44 - protein, 9 aa, synthetic construct
  VARIANT 1: note = ACE
  VARIANT 2: note = M3L
  VARIANT 9: note = NME
XXAAAGHKX

SEQ ID NO: 45-49 - skipped (5 entries)

SEQ ID NO: 50 - protein, 9 aa, synthetic construct
  VARIANT 1: note = ACE
  VARIANT 2: note = M3L
  VARIANT 9: note = NME
XXGGGGHKX

SEQ ID NO: 51-53 - skipped (3 entries)

SEQ ID NO: 54 - protein, 9 aa, synthetic construct
  VARIANT 1: note = ACE
  VARIANT 2: note = 4PH
  VARIANT 9: note = NME
XXAAAGHKX

SEQ ID NO: 55-59 - skipped (5 entries)

SEQ ID NO: 60 - protein, 9 aa, synthetic construct
  VARIANT 1: note = ACE
  VARIANT 2: note = 4PH
  VARIANT 9: note = NME
XXGGGGHKX

SEQ ID NO: 61-63 - skipped (3 entries)

SEQ ID NO: 64 - protein, 9 aa, synthetic construct
  VARIANT 1: note = ACE
  VARIANT 5: note = M3L
  VARIANT 9: note = NME
XAAAXGHKX

SEQ ID NO: 65-69 - skipped (5 entries)

SEQ ID NO: 70 - protein, 9 aa, synthetic construct
  VARIANT 1: note = ACE
  VARIANT 5: note = M3L
  VARIANT 9: note = NME
XGGGXGHKX

SEQ ID NO: 71-73 - skipped (3 entries)

SEQ ID NO: 74 - protein, 8 aa, synthetic construct
  VARIANT 1: note = ACE
  VARIANT 8: note = NME
XAAAKHGX

SEQ ID NO: 75-79 - skipped (5 entries)

SEQ ID NO: 80 - protein, 8 aa, synthetic construct
  VARIANT 1: note = ACE
  VARIANT 8: note = NME
XGGGKHGX

SEQ ID NO: 81-83 - skipped (3 entries)

SEQ ID NO: 84 - protein, 9 aa, synthetic construct
  VARIANT 1: note = ACE
  VARIANT 2: note = M3L
  VARIANT 9: note = NME
XXAAAKHGX

SEQ ID NO: 85-89 - skipped (5 entries)

SEQ ID NO: 90 - protein, 9 aa, synthetic construct
  VARIANT 1: note = ACE
  VARIANT 2: note = M3L
  VARIANT 9: note = NME
XXGGGKHGX

SEQ ID NO: 91-93 - skipped (3 entries)

SEQ ID NO: 94 - protein, 10 aa, synthetic construct
  VARIANT 1: note = ACE
  VARIANT 2: note = 4PH
  VARIANT 3: note = M3L
  VARIANT 10: note = NME
XXXAAAGHKX

SEQ ID NO: 95-99 - skipped (5 entries)

SEQ ID NO: 100 - protein, 10 aa, synthetic construct
  VARIANT 1: note = ACE
  VARIANT 2: note = 4PH
  VARIANT 3: note = M3L
  VARIANT 10: note = NME
XXXGGGGHKX

SEQ ID NO: 101-103 - skipped (3 entries)

SEQ ID NO: 104 - protein, 10 aa, synthetic construct
  VARIANT 1: note = ACE
  VARIANT 2: note = ZCL
  VARIANT 3: note = M3L
  VARIANT 10: note = NME
XXXAAAGHKX

SEQ ID NO: 105-109 - skipped (5 entries)

SEQ ID NO: 110 - protein, 10 aa, synthetic construct
  VARIANT 1: note = ACE
  VARIANT 2: note = ZCL
  VARIANT 3: note = M3L
  VARIANT 10: note = NME
XXXGGGGHKX

SEQ ID NO: 111-113 - skipped (3 entries)

SEQ ID NO: 114 - protein, 10 aa, synthetic construct
  VARIANT 1: note = ACE
  VARIANT 2: note = A30
  VARIANT 3: note = M3L
  VARIANT 10: note = NME
XXXAAAGHKX

SEQ ID NO: 115-119 - skipped (5 entries)

SEQ ID NO: 120 - protein, 10 aa, synthetic construct
  VARIANT 1: note = ACE
  VARIANT 2: note = A30
  VARIANT 3: note = M3L
  VARIANT 10: note = NME
XXXGGGGHKX

SEQ ID NO: 121-123 - skipped (3 entries)

SEQ ID NO: 124 - protein, 9 aa, synthetic construct
  VARIANT 1: note = ACE
  VARIANT 8: note = 4PH
  VARIANT 9: note = NME
XAAAGHKXX

SEQ ID NO: 125-129 - skipped (5 entries)

SEQ ID NO: 130 - protein, 9 aa, synthetic construct
  VARIANT 1: note = ACE
  VARIANT 8: note = 4PH
  VARIANT 9: note = NME
XGGGGHKXX

SEQ ID NO: 131 - protein, 8 aa, synthetic construct
  VARIANT 1: note = ACE
  VARIANT 2: note = P15
  VARIANT 7: note = 4PH
  VARIANT 8: note = NME
XXGHKGXX

SEQ ID NO: 132 - protein, 8 aa, synthetic construct
  VARIANT 1: note = ACE
  VARIANT 2: note = P10
  VARIANT 7: note = 4PH
  VARIANT 8: note = NME
XXGHKGXX

SEQ ID NO: 133 - protein, 8 aa, synthetic construct
  VARIANT 1: note = ACE
  VARIANT 2: note = P13
  VARIANT 7: note = 4PH
  VARIANT 8: note = NME
XXGHKGXX

SEQ ID NO: 134 - protein, 10 aa, synthetic construct
  VARIANT 1: note = ACE
  VARIANT 9: note = 4PH
  VARIANT 10: note = NME
XAAAGHKGXX

SEQ ID NO: 135 - protein, 8 aa, synthetic construct
  VARIANT 1: note = ACE
  VARIANT 2: note = P11
  VARIANT 7: note = 4PH
  VARIANT 8: note = NME
XXGHKGXX

SEQ ID NO: 136 - protein, 8 aa, synthetic construct
  VARIANT 1: note = ACE
  VARIANT 2: note = P21
  VARIANT 7: note = 4PH
  VARIANT 8: note = NME
XXGHKGXX

SEQ ID NO: 137 - protein, 8 aa, synthetic construct
  VARIANT 1: note = ACE
  VARIANT 2: note = P06
  VARIANT 7: note = 4PH
  VARIANT 8: note = NME
XXGHKGXX

SEQ ID NO: 138 - protein, 8 aa, synthetic construct
  VARIANT 1: note = ACE
  VARIANT 2: note = P12
  VARIANT 7: note = 4PH
  VARIANT 8: note = NME
XXGHKGXX

SEQ ID NO: 139 - protein, 8 aa, synthetic construct
  VARIANT 1: note = ACE
  VARIANT 2: note = P14
  VARIANT 7: note = 4PH
  VARIANT 8: note = NME
XXGHKGXX

SEQ ID NO: 140 - protein, 10 aa, synthetic construct
  VARIANT 1: note = ACE
  VARIANT 9: note = 4PH
  VARIANT 10: note = NME
XGGGGHKGXX

SEQ ID NO: 141 - protein, 8 aa, synthetic construct
  VARIANT 1: note = ACE
  VARIANT 2: note = P15
  VARIANT 7: note = 4PH
  VARIANT 8: note = NME
XXGHKAXX

SEQ ID NO: 142 - protein, 8 aa, synthetic construct
  VARIANT 1: note = ACE
  VARIANT 2: note = P10
  VARIANT 7: note = 4PH
  VARIANT 8: note = NME
XXGHKAXX

SEQ ID NO: 143 - protein, 8 aa, synthetic construct
  VARIANT 1: note = ACE
  VARIANT 2: note = P13
  VARIANT 7: note = 4PH
  VARIANT 8: note = NME
XXGHKAXX

SEQ ID NO: 144 - protein, 10 aa, synthetic construct
  VARIANT 1: note = ACE
  VARIANT 9: note = 4PH
  VARIANT 10: note = NME
XAAAGHKAXX

SEQ ID NO: 145 - protein, 8 aa, synthetic construct
  VARIANT 1: note = ACE
  VARIANT 2: note = P11
  VARIANT 7: note = 4PH
  VARIANT 8: note = NME
XXGHKAXX

SEQ ID NO: 146 - protein, 8 aa, synthetic construct
  VARIANT 1: note = ACE
  VARIANT 2: note = P21
  VARIANT 7: note = 4PH
  VARIANT 8: note = NME
XXGHKAXX

SEQ ID NO: 147 - protein, 8 aa, synthetic construct
  VARIANT 1: note = ACE
  VARIANT 2: note = P06
  VARIANT 7: note = 4PH
  VARIANT 8: note = NME
XXGHKAXX

SEQ ID NO: 148 - protein, 8 aa, synthetic construct
  VARIANT 1: note = ACE
  VARIANT 2: note = P12
  VARIANT 7: note = 4PH
  VARIANT 8: note = NME
XXGHKAXX

SEQ ID NO: 149 - protein, 8 aa, synthetic construct
  VARIANT 1: note = ACE
  VARIANT 2: note = P14
  VARIANT 7: note = 4PH
  VARIANT 8: note = NME
XXGHKAXX

SEQ ID NO: 150 - protein, 10 aa, synthetic construct
  VARIANT 1: note = ACE
  VARIANT 9: note = 4PH
  VARIANT 10: note = NME
XGGGGHKAXX

SEQ ID NO: 151 - protein, 9 aa, synthetic construct
  VARIANT 1: note = ACE
  VARIANT 2: note = M3L
  VARIANT 3: note = P15
  VARIANT 8: note = 4PH
  VARIANT 9: note = NME
XXXGHKAXX

SEQ ID NO: 152 - protein, 9 aa, synthetic construct
  VARIANT 1: note = ACE
  VARIANT 2: note = M3L
  VARIANT 3: note = P10
  VARIANT 8: note = 4PH
  VARIANT 9: note = NME
XXXGHKAXX

SEQ ID NO: 153 - protein, 9 aa, synthetic construct
  VARIANT 1: note = ACE
  VARIANT 2: note = M3L
  VARIANT 3: note = P13
  VARIANT 8: note = 4PH
  VARIANT 9: note = NME
XXXGHKAXX

SEQ ID NO: 154 - protein, 11 aa, synthetic construct
  VARIANT 1: note = ACE
  VARIANT 2: note = M3L
  VARIANT 10: note = 4PH
  VARIANT 11: note = NME
XXAAAGHKAXX

SEQ ID NO: 155 - protein, 9 aa, synthetic construct
  VARIANT 1: note = ACE
  VARIANT 2: note = M3L
  VARIANT 3: note = P11
  VARIANT 8: note = 4PH
  VARIANT 9: note = NME
XXXGHKAXX

SEQ ID NO: 156 - protein, 9 aa, synthetic construct
  VARIANT 1: note = ACE
  VARIANT 2: note = M3L
  VARIANT 3: note = P21
  VARIANT 8: note = 4PH
  VARIANT 9: note = NME
XXXGHKAXX

SEQ ID NO: 157 - protein, 9 aa, synthetic construct
  VARIANT 1: note = ACE
  VARIANT 2: note = M3L
  VARIANT 3: note = P06
  VARIANT 8: note = 4PH
  VARIANT 9: note = NME
XXXGHKAXX

SEQ ID NO: 158 - protein, 9 aa, synthetic construct
  VARIANT 1: note = ACE
  VARIANT 2: note = M3L
  VARIANT 3: note = P12
  VARIANT 8: note = 4PH
  VARIANT 9: note = NME
XXXGHKAXX

SEQ ID NO: 159 - protein, 9 aa, synthetic construct
  VARIANT 1: note = ACE
  VARIANT 2: note = M3L
  VARIANT 3: note = P14
  VARIANT 8: note = 4PH
  VARIANT 9: note = NME
XXXGHKAXX

SEQ ID NO: 160 - protein, 11 aa, synthetic construct
  VARIANT 1: note = ACE
  VARIANT 2: note = M3L
  VARIANT 10: note = 4PH
  VARIANT 11: note = NME
XXGGGGHKAXX

SEQ ID NO: 161-163 - skipped (3 entries)

SEQ ID NO: 164 - protein, 8 aa, synthetic construct
  SITE 6: note = D-Histidine
  VARIANT 1: note = ACE
  SITE 7: note = D-Lysine
  VARIANT 8: note = NME
XAAAGHKX

SEQ ID NO: 165-169 - skipped (5 entries)

SEQ ID NO: 170 - protein, 8 aa, synthetic construct
  VARIANT 1: note = ACE
  SITE 6: note = D-Histidine
  SITE 7: note = D-Lysine
  VARIANT 8: note = NME
XGGGGHKX

SEQ ID NO: 171-173 - skipped (3 entries)

SEQ ID NO: 174 - protein, 9 aa, synthetic construct
  VARIANT 1: note = ACE
  VARIANT 2: note = M3L
  VARIANT 9: note = NME
  SITE 7: note = D-Histidine
  SITE 8: note = D-Lysine
XXAAAGHKX

SEQ ID NO: 175-179 - skipped (5 entries)

SEQ ID NO: 180 - protein, 9 aa, synthetic construct
  VARIANT 1: note = ACE
  VARIANT 2: note = M3L
  SITE 7: note = D-Histidine
  SITE 8: note = D-Lysine
  VARIANT 9: note = NME
XXGGGGHKX

SEQ ID NO: 181-183 - skipped (3 entries)

SEQ ID NO: 184 - protein, 8 aa, synthetic construct
  VARIANT 1: note = ACE
  VARIANT 7: note = LYO
  VARIANT 8: note = NME
XAAAGHXX

SEQ ID NO: 185-189 - skipped (5 entries)

SEQ ID NO: 190 - protein, 8 aa, synthetic construct
  VARIANT 1: note = ACE
  VARIANT 7: note = LYO
  VARIANT 8: note = NME
XGGGGHXX

SEQ ID NO: 191-193 - skipped (3 entries)

SEQ ID NO: 194 - protein, 9 aa, synthetic construct
  VARIANT 1: note = ACE
  VARIANT 2: note = M3L
  VARIANT 8: note = LYO
  VARIANT 9: note = NME
XXAAAGHXX

SEQ ID NO: 195-199 - skipped (5 entries)

SEQ ID NO: 200 - protein, 9 aa, synthetic construct
  VARIANT 1: note = ACE
  VARIANT 2: note = M3L
  VARIANT 8: note = LYO
  VARIANT 9: note = NME
XXGGGGHXX

SEQ ID NO: 201-203 - skipped (3 entries)

SEQ ID NO: 204 - protein, 8 aa, synthetic construct
  VARIANT 1: note = ACE
  VARIANT 7: note = LHY
  VARIANT 8: note = NME
XAAAGHXX

SEQ ID NO: 205-209 - skipped (5 entries)

SEQ ID NO: 210 - protein, 8 aa, synthetic construct
  VARIANT 1: note = ACE
  VARIANT 7: note = LHY
  VARIANT 8: note = NME
XGGGGHXX

SEQ ID NO: 211-213 - skipped (3 entries)

SEQ ID NO: 214 - protein, 9 aa, synthetic construct
  VARIANT 1: note = ACE
  VARIANT 2: note = M3L
  VARIANT 8: note = LHY
  VARIANT 9: note = NME
XXAAAGHXX

SEQ ID NO: 215-219 - skipped (5 entries)

SEQ ID NO: 220 - protein, 9 aa, synthetic construct
  VARIANT 1: note = ACE
  VARIANT 2: note = M3L
  VARIANT 8: note = LHY
  VARIANT 9: note = NME
XXGGGGHXX

SEQ ID NO: 221-233 - skipped (13 entries)

SEQ ID NO: 234 - protein, 9 aa, synthetic construct
  VARIANT 1: note = PAL
  VARIANT 2: note = M3L
  VARIANT 9: note = OH
XXAAAGHKX

SEQ ID NO: 235-236 - skipped (2 entries)

SEQ ID NO: 237 - protein, 9 aa, synthetic construct
  VARIANT 1: note = PAL
  VARIANT 2: note = M3L
  SITE 7: note = D-Histidine
  SITE 8: note = D-Lysine
  VARIANT 9: note = OH
XXAAAGHKX

SEQ ID NO: 238-257 - skipped (20 entries)

SEQ ID NO: 258 - protein, 8 aa, synthetic construct
  VARIANT 1: note = PAL
  VARIANT 7: note = LHY
  VARIANT 8: note = OH
XAAAGHXX

SEQ ID NO: 259 - protein, 8 aa, synthetic construct
  VARIANT 1: note = PAL
  VARIANT 7: note = LHY
  VARIANT 8: note = OH
XGGGGHXX

SEQ ID NO: 260-268 - skipped (9 entries)

SEQ ID NO: 269 - protein, 7 aa, synthetic construct
  VARIANT 1: note = ACE
  VARIANT 7: note = NME
XGGGHKX

SEQ ID NO: 270 - protein, 7 aa, synthetic construct
  VARIANT 1: note = ACE
  VARIANT 7: note = NME
XAAGHKX

SEQ ID NO: 271 - protein, 7 aa, synthetic construct
  VARIANT 1: note = ACE
  VARIANT 7: note = NME
XPPGHKX

SEQ ID NO: 272 - protein, 8 aa, synthetic construct
  VARIANT 1: note = ACE
  VARIANT 8: note = NME
XPPPGHKX

SEQ ID NO: 273-276 - skipped (4 entries)

SEQ ID NO: 277 - protein, 8 aa, synthetic construct
  VARIANT 1: note = ACE
  VARIANT 2: note = M3L
  VARIANT 8: note = NME
XXGGGHKX

SEQ ID NO: 278 - protein, 8 aa, synthetic construct
  VARIANT 1: note = ACE
  VARIANT 2: note = M3L
  VARIANT 8: note = NME
XXAAGHKX

SEQ ID NO: 279 - protein, 8 aa, synthetic construct
  VARIANT 1: note = ACE
  VARIANT 2: note = M3L
  VARIANT 8: note = NME
XXPPGHKX

SEQ ID NO: 280 - protein, 9 aa, synthetic construct
  VARIANT 1: note = ACE
  VARIANT 2: note = M3L
  VARIANT 9: note = NME
XXPPPGHKX

SEQ ID NO: 281 - skipped

SEQ ID NO: 282 - protein, 9 aa, synthetic construct
  VARIANT 1: note = ACE
  VARIANT 2: note = 4PH
  VARIANT 9: note = NME
XXPPPGHKX

SEQ ID NO: 283 - skipped

SEQ ID NO: 284 - protein, 9 aa, synthetic construct
  VARIANT 1: note = ACE
  VARIANT 5: note = M3L
  VARIANT 9: note = NME
XPPPXGHKX

SEQ ID NO: 285 - skipped

SEQ ID NO: 286 - protein, 8 aa, synthetic construct
  VARIANT 1: note = ACE
  VARIANT 8: note = NME
XPPPKHGX

SEQ ID NO: 287 - skipped

SEQ ID NO: 288 - protein, 9 aa, synthetic construct
  VARIANT 1: note = ACE
  VARIANT 2: note = M3L
  VARIANT 9: note = NME
XXPPPKHGX

SEQ ID NO: 289 - skipped

SEQ ID NO: 290 - protein, 8 aa, synthetic construct
  VARIANT 1: note = ACE
  SITE 6: note = D-Histidine
  SITE 7: note = D-Lysine
  VARIANT 8: note = NME
XPPPGHKX

SEQ ID NO: 291 - skipped

SEQ ID NO: 292 - protein, 9 aa, synthetic construct
  VARIANT 1: note = ACE
  VARIANT 2: note = M3L
  SITE 7: note = D-Histidine
  SITE 8: note = D-Lysine
  VARIANT 9: note = NME
XXPPPGHKX

SEQ ID NO: 293 - skipped

SEQ ID NO: 294 - protein, 8 aa, synthetic construct
  VARIANT 1: note = PAL
  VARIANT 8: note = OH
XPPPGHKX

SEQ ID NO: 295 - skipped

SEQ ID NO: 296 - protein, 8 aa, synthetic construct
  VARIANT 1: note = BIO
  VARIANT 8: note = NH2
XPPPGHKX

SEQ ID NO: 297-336 - skipped (40 entries)

SEQ ID NO: 337 - protein, 8 aa, synthetic construct
  VARIANT 1: note = ACE
  VARIANT 2: note = M3L
  VARIANT 7: note = 4PH
  VARIANT 8: note = NME
XXGHKAXX

SEQ ID NO: 338 - protein, 8 aa, synthetic construct
  VARIANT 1: note = ACE
  VARIANT 2: note = M3L
  VARIANT 7: note = ZCL
  VARIANT 8: note = NME
XXGHKAXX

SEQ ID NO: 339 - protein, 8 aa, synthetic construct
  VARIANT 1: note = ACE
  VARIANT 2: note = M3L
  VARIANT 7: note = A30
  VARIANT 8: note = NME
XXGHKAXX

SEQ ID NO: 340 - protein, 9 aa, synthetic construct
  VARIANT 1: note = ACE
  VARIANT 2: note = M3L
  VARIANT 3: note = 2MR
  VARIANT 8: note = 4PH
  VARIANT 9: note = NME
XXXGHKAXX

SEQ ID NO: 341 - protein, 9 aa, synthetic construct
  VARIANT 1: note = ACE
  VARIANT 2: note = M3L
  VARIANT 3: note = 2MR
  VARIANT 8: note = ZCL
  VARIANT 9: note = NME
XXXGHKAXX

SEQ ID NO: 342 - protein, 9 aa, synthetic construct
  VARIANT 1: note = ACE
  VARIANT 2: note = M3L
  VARIANT 3: note = 2MR
  VARIANT 8: note = A30
  VARIANT 9: note = NME
XXXGHKAXX

SEQ ID NO: 343 - protein, 9 aa, synthetic construct
  VARIANT 1: note = ACE
  VARIANT 2: note = 2MR
  VARIANT 3: note = M3L
  VARIANT 8: note = 4PH
  VARIANT 9: note = NME
XXXGHKAXX

SEQ ID NO: 344 - protein, 9 aa, synthetic construct
  VARIANT 1: note = ACE
  VARIANT 2: note = 2MR
  VARIANT 3: note = M3L
  VARIANT 8: note = ZCL
  VARIANT 9: note = NME
XXXGHKAXX

SEQ ID NO: 345 - protein, 9 aa, synthetic construct
  VARIANT 1: note = ACE
  VARIANT 2: note = 2MR
  VARIANT 3: note = M3L
  VARIANT 8: note = A30
  VARIANT 9: note = NME
XXXGHKAXX

SEQ ID NO: 346-348 - skipped (3 entries)

SEQ ID NO: 349 - protein, 8 aa, synthetic construct
  VARIANT 1: note = ACE
  VARIANT 2: note = M3L
  VARIANT 7: note = 4PH
  VARIANT 8: note = NME
XXGHKGXX

SEQ ID NO: 350 - protein, 8 aa, synthetic construct
  VARIANT 1: note = ACE
  VARIANT 2: note = M3L
  VARIANT 7: note = ZCL
  VARIANT 8: note = NME
XXGHKGXX

SEQ ID NO: 351 - protein, 8 aa, synthetic construct
  VARIANT 1: note = ACE
  VARIANT 2: note = M3L
  VARIANT 7: note = A30
  VARIANT 8: note = NME
XXGHKGXX

SEQ ID NO: 352 - protein, 8 aa, synthetic construct
  VARIANT 1: note = ACE
  VARIANT 2: note = M3L
  VARIANT 7: note = 4PH
  VARIANT 8: note = NME
XXGHKPXX

SEQ ID NO: 353 - protein, 8 aa, synthetic construct
  VARIANT 1: note = ACE
  VARIANT 2: note = M3L
  VARIANT 7: note = ZCL
  VARIANT 8: note = NME
XXGHKPXX

SEQ ID NO: 354 - protein, 8 aa, synthetic construct
  VARIANT 1: note = ACE
  VARIANT 2: note = M3L
  VARIANT 7: note = A30
  VARIANT 8: note = NME
XXGHKPXX

SEQ ID NO: 355-408 - skipped (54 entries)

SEQ ID NO: 409 - protein, 8 aa, synthetic construct
  VARIANT 1: note = ACE
  VARIANT 2: note = 4PH
  VARIANT 7: note = M3L
  VARIANT 8: note = NME
XXAKHGXX

SEQ ID NO: 410 - protein, 8 aa, synthetic construct
  VARIANT 1: note = ACE
  VARIANT 2: note = ZCL
  VARIANT 7: note = M3L
  VARIANT 8: note = NME
XXAKHGXX

SEQ ID NO: 411 - protein, 8 aa, synthetic construct
  VARIANT 1: note = ACE
  VARIANT 2: note = A30
  VARIANT 7: note = M3L
  VARIANT 8: note = NME
XXAKHGXX

SEQ ID NO: 412 - protein, 8 aa, synthetic construct
  VARIANT 1: note = ACE
  VARIANT 2: note = 4PH
  VARIANT 7: note = M3L
  VARIANT 8: note = NME
XXGKHGXX

SEQ ID NO: 413 - protein, 8 aa, synthetic construct
  VARIANT 1: note = ACE
  VARIANT 2: note = ZCL
  VARIANT 7: note = M3L
  VARIANT 8: note = NME
XXGKHGXX

SEQ ID NO: 414 - protein, 8 aa, synthetic construct
  VARIANT 1: note = ACE
  VARIANT 2: note = A30
  VARIANT 7: note = M3L
  VARIANT 8: note = NME
XXGKHGXX

SEQ ID NO: 415 - protein, 8 aa, synthetic construct
  VARIANT 1: note = PAL
  VARIANT 2: note = 4PH
  VARIANT 7: note = M3L
  VARIANT 8: note = OH
XXAKHGXX

SEQ ID NO: 416 - protein, 8 aa, synthetic construct
  VARIANT 1: note = PAL
  VARIANT 2: note = ZCL
  VARIANT 7: note = M3L
  VARIANT 8: note = OH
XXAKHGXX

SEQ ID NO: 417 - protein, 8 aa, synthetic construct
  VARIANT 1: note = PAL
  VARIANT 2: note = A30
  VARIANT 7: note = M3L
  VARIANT 8: note = OH
XXAKHGXX

SEQ ID NO: 418 - protein, 8 aa, synthetic construct
  VARIANT 1: note = BIO
  VARIANT 2: note = 4PH
  VARIANT 7: note = M3L
  VARIANT 8: note = NH2
XXAKHGXX

SEQ ID NO: 419 - protein, 8 aa, synthetic construct
  VARIANT 1: note = BIO
  VARIANT 2: note = ZCL
  VARIANT 7: note = M3L
  VARIANT 8: note = NH2
XXAKHGXX

SEQ ID NO: 420 - protein, 8 aa, synthetic construct
  VARIANT 1: note = BIO
  VARIANT 2: note = A30
  VARIANT 7: note = M3L
  VARIANT 8: note = NH2
XXAKHGXX

SEQ ID NO: 421-423 - skipped (3 entries)

SEQ ID NO: 424 - protein, 8 aa, synthetic construct
  VARIANT 1: note = PAL
  VARIANT 2: note = M3L
  VARIANT 7: note = 4PH
  VARIANT 8: note = OH
XXGHKAXX

SEQ ID NO: 425 - protein, 8 aa, synthetic construct
  VARIANT 1: note = PAL
  VARIANT 2: note = M3L
  VARIANT 7: note = ZCL
  VARIANT 8: note = OH
XXGHKAXX

SEQ ID NO: 426 - protein, 8 aa, synthetic construct
  VARIANT 1: note = PAL
  VARIANT 2: note = M3L
  VARIANT 7: note = A30
  UNSURE 8: note = OH
XXGHKAXX

SEQ ID NO: 427 - protein, 8 aa, synthetic construct
  VARIANT 1: note = PAL
  VARIANT 2: note = MLZ
  VARIANT 7: note = 4PH
  VARIANT 8: note = OH
XXGHKAXX

SEQ ID NO: 428 - protein, 8 aa, synthetic construct
  VARIANT 1: note = PAL
  VARIANT 2: note = MLZ
  VARIANT 7: note = ZCL
  VARIANT 8: note = OH
XXGHKAXX

SEQ ID NO: 429 - protein, 8 aa, synthetic construct
  VARIANT 1: note = PAL
  VARIANT 2: note = MLZ
  VARIANT 7: note = A30
  VARIANT 8: note = OH
XXGHKAXX

SEQ ID NO: 430 - protein, 8 aa, synthetic construct
  VARIANT 1: note = PAL
  VARIANT 2: note = MLY
  VARIANT 7: note = 4PH
  VARIANT 8: note = OH
XXGHKAXX

SEQ ID NO: 431 - protein, 8 aa, synthetic construct
  VARIANT 1: note = PAL
  VARIANT 2: note = MLY
  VARIANT 7: note = ZCL
  VARIANT 8: note = OH
XXGHKAXX

SEQ ID NO: 432 - protein, 8 aa, synthetic construct
  VARIANT 1: note = PAL
  VARIANT 2: note = MLY
  VARIANT 7: note = A30
  VARIANT 8: note = OH
XXGHKAXX

SEQ ID NO: 433 - protein, 9 aa, synthetic construct
  source 1..9: note; note (original language) = 式I-a
  VARIANT 1: note = R1
  VARIANT 5: note = L2
  VARIANT 9: note = R2
XGHKXGHKX